European Patent Application EP 4 459 287 A1, published November 6, 2024. Title: METHODS AND TOOLS FOR DETECTING THE IMPACT OF COMPOUNDS ON PROTEIN, RNA OR DNA INTERACTIONS. Applicant: SYNSIGHT. Application EP. The sequence listing filed with the application follows.

SEQUENCE LISTING (23 sequences)

SEQ ID NO: 1 - protein, 449 aa, Homo sapiens
MRECISIHVGQAGVQIGNACWELYCLEHGIQPDGQMPSDKTIGGGDDSFNTFFSETGAGKHVPRAVFVDLEPTVIDEVRTGTYRQLFHPEQLITGKEDAANYARGHYTIGKEIIDLVLDRIRKLADQCTRLQGFLVFHSFGGGTGSGFTSLLMERLSVDYGKSKLEFSIYPAPQVSTAVVEPYNSILTTHTTLEHSDCAFMVDNEAIYDICRRNLDIERPTYTNLNRLISQIVSSITASLRFDGALNVDLTEFQTNLVPYPRIHFPLATYAPVISAEKAYHEQLSVADITNACFEPANQMVKCDPGHGKYMACCLLYRGDVVPKDVNAAIATIKTKRTIQFVDWCPTGFKVGINYQPPTVVPGGDLAKVQRAVCMLSNTTAIAEAWARLDHKFDLMYAKRAFVHWYVGEGMEEGEFSEAREDMAALEKDYEEVGVDSVEGEGEEEGEEY

SEQ ID NO: 2 - protein, 440 aa, Homo sapiens
MREIVHIQAGQCGNQIGAKFWEVISDEHGIDPTGTYHGDSDLQLDRISVYYNEATGGKYVPRAILVDLEPGTMDSVRSGPFGQIFRPDNFVFGQSGAGNWAKGHYTEGAELVDSVLDVVRKEAESCDCLQGFQLTHSLGGGTGSGMGTLLISKIREEYPDRIMNTFSVVPSPKVSDTVVEPYNATLSVHQLVENTDETYCIDNEALYDICFRTLRLTTPTYGDLNHLVSGTMECVTTCLRFPGQLNADLRKLAVNMVPFPRLHFFMPGFAPLTSRGSQQYRALTVPDLTQQVFDAKMMAACDPRHGRYLTVAAVFRGRMSMKEVDEQMLNVQNKSSYFVEWIPNVKTAVCDIPPRGLKMAVTFIGNSTAIQELFKRISEQFTAMFRRKAFLHWYTGEGMDEMEFTEAESNMNDLVSEYQQYQDATAEEEEDFGEEAEEEA

SEQ ID NO: 3 - protein, 150 aa, Homo sapiens
MAEPRQEFEVMEDHAGTYGLGDRKDQGGYTMHQDQEGDTDAGLKESPLQTPTEDGSEEPGSETSDAKSTPTAEDVTAPLVDEGAPGKQAAAQPHTEIPEGTTAEEAGIGDTPSLEDEAAGHVTQARMVSKSKDGTGSDDKKAKGADGKTK

SEQ ID NO: 4 - protein, 248 aa, Homo sapiens
IATPRGAAPPGQKGQANATRIPAKTPPAPKTPPSSGEPPKSGDRSGYSSPGSPGTPGSRSRTPSLPTPPTREPKVAVVRTPPKSPSSAKSRLQTAPVPMPDLKVKSKIGSTENLKHQPGGGKVQIINKKLDLSNVQSKCGSKDNIKHVPGGGSVQIVYKPVDLSKVTSKCGSLGNIHHKPGGGQVEVKSEKLDFKDRVQSKIGSLDNITHVPGGGNKKIETHKLTFRENAKAKTDHGAEIVYKSPVVS

SEQ ID NO: 5 - protein, 32 aa, Homo sapiens
LQTAPVPMPDLKNVKSKIGSTENLKHQPGGGK

SEQ ID NO: 6 - protein, 31 aa, Homo sapiens
VQIINKKLDLSNVQSKCGSKDNIKHVPGGGS

SEQ ID NO: 7 - protein, 31 aa, Homo sapiens
VQIVYKPVDLSKVTSKCGSLGNIHHKPGGGQ

SEQ ID NO: 8 - protein, 32 aa, Homo sapiens
VEVKSEKLDFKDRVQSKIGSLDNITHVPGGGN

SEQ ID NO: 9 - protein, 357 aa, Homo sapiens
QNKILEGLEKLRHLDFLRYPVATQKDLASGAVPTNLKPSKIKQRADSKESLKATTKTAVSKLAKREEVVEEGAKEARSELAKELAKTEKKAKESSEKPPEKPAKPERVKTESSEALKAEKRKLIKDKVGKKHLKEKISKLEEKKDKEKKEIKERKELKKDEGRKEEKKDAKKEEKRKDTKPELKKISKPDLKPFTPEVRKTLYKAKVPGRVKIDRSRAIRGEKELSSEPQTPPAQKGTVPLPTISGHRELVLSSPEDLTQDFEEMKREERALLAEQRDTGLGDKPFPLDTAEEGPPSTAIQGTPPSVPGLGQEEHVMKEKELVPEVPEEQGSKDRGLDSGAETEEEKDTWEEKKQRE

SEQ ID NO: 10 - protein, 305 aa, Homo sapiens
FKQAKDKVSDGVTKSPEKRSSLPRPSSILPPRRGVSGDRDENSFSLNSSISSSARRTTRSEPIRRAGKSGTSTPTTPGSTAITPGTPPSYSSRTPGTPGTPSYPRTPHTPGTPKSAILVPSEKVAIIRTPPKSPATPKQLRLINQPLPDLKVKSKIGSTDNIKYQPKGGQVQIVTKKIDLSHVTSKCGSLKIRHRPGGGRVKIESVKLDFKEKAQAKVGSLDNAHHVPGGGNVKIDSQKLNFREHAKARVDHGAEIITQSPGRSSVASPRRLSNVSSSGSINLLESPQLATLAEDVTAALAKQGL

SEQ ID NO: 11 - protein, 158 aa, Homo sapiens
LATNTSAPDLKVRSKVGSTENIKHQPGGGRAKVEKTEAAATTRKPESNAVTKTAGPIASAQKQPAGKVQIVSKVSYSHIQSKCGSKDNIKHVPGGGNVQIQNKVDISKVSSKCGSKANIKHKPGGGDVKIESQKLNFKEKAQAKVGSLDNVGHLPAGG

SEQ ID NO: 12 - protein, 203 aa, Homo sapiens
SVMRQDYRAWKVQRPEPSCRPRSEYQPSDAPFERETQYQKDFRAWPLPRRGDHPWIPKPVQISAASQASAPILGAPKRRPQSQERWPVQAAAEAREQEAAPGGAGGLAAGKASGADERDTRRKAGPAWIVRRAEGLGHEQTPLPAAQAQVQATGPEAGRGRAAADALNRQIREEVASAVSSSYRNEFRAWTDIKPVKPIKAKP

SEQ ID NO: 13 - protein, 144 aa, Homo sapiens
YDPVAARQGQETAVAPSLVAPALNKPKKPLTSSSAAPQRPISTQRTAAAPKAGPGVVRKPGVGNGDDEAAELMQQVNVLKLTVEDLEKERDFYFGKLRNIELICQENEGENDPVLQRIVDILYATDEGFVIPDEGGPQEEQEEY

SEQ ID NO: 14 - protein, 441 aa, Homo sapiens
MAEPRQEFEVMEDHAGTYGLGDRKDQGGYTMHQDQEGDTDAGLKESPLQTPTEDGSEEPGSETSDAKSTPTAEDVTAPLVDEGAPGKQAAAQPHTEIPEGTTAEEAGIGDTPSLEDEAAGHVTQARMVSKSKDGTGSDDKKAKGADGKTKIATPRGAAPPGQKGQANATRIPAKTPPAPKTPPSSGEPPKSGDRSGYSSPGSPGTPGSRSRTPSLPTPPTREPKKVAVVRTPPKSPSSAKSRLQTAPVPMPDLKNVKSKIGSTENLKHQPGGGKVQIINKKLDLSNVQSKCGSKDNIKHVPGGGSVQIVYKPVDLSKVTSKCGSLGNIHHKPGGGQVEVKSEKLDFKDRVQSKIGSLDNITHVPGGGNKKIETHKLTFRENAKAKTDHGAEIVYKSPVVSGDTSPRHLSNVSSTGSIDMVDSPQLATLADEVSASLAKQGL

SEQ ID NO: 15 - protein, 393 aa, Homo sapiens [sequence omitted]

SEQ ID NO: 16 - protein, 393 aa, Homo sapiens
MEEPQSDPSVEPPLSQETFSDLAKLLPENNVLSPLPSQAMDDLMLSPDDIEQWFTEDPGPDEAPRMPEAAPPVAPAPAAPTPAAPAPAPSWPLSSSVPSQKTYQGSYGFRLGFLHSGTAKSVTCTYSPALNKMFCQLAKTCPVQLWVDSTPPPGTRVRAMAIYKQSQHMTEVVRRCPHHERCSDSDGLAPPQHLIRVEGNLRVEYLDDRNTFRHSVVVPYEPPEVGSDCTTIHYNYMCNSSCMGGMNRRPILTIITLEDSSGNLLGRNSFEVRVCACPGRDRRTEEENLRKKGEPHHELPPGSTKRALPNNTSSSPQPKKKPLDGEYFTLQIRGRERFEMFRELNEALELKDAQAGKEPGGSRAHSSHLKSKKGQSTSRHKKLMFKTEGPDSD

SEQ ID NO: 17 - protein, 314 aa, Homo sapiens
MEEPQSDPSVEPPLSQETASDLWKLLPENNVLSPLPSQAMDDLMLSPDDIEQWFTEDPGPDEAPRMPEAAPPVAPAPAAPTPAAPAPAPSWPLSSSVPSQKTYQGSYGFRLGFLHSGTAKSVTCTYSPALNKMFCQLAKTCPVQLWVDSTPPPGTRVRAMAIYKQSQHMTEVVRRCPHHERCSDSDGLAPPQHLIRVEGNLRVEYLDDRNTFRHSVVVPYEPPEVGSDCTTIHYNYMCNSSCMGGMNRRPILTIITLEDSSGNLLGRNSFEVRVCACPGRDRRTEEENLRKKGEPHHELPPGSTKRALPNNTSS

SEQ ID NO: 18 - protein, 393 aa, Homo sapiens
MEEPQSDPSVEPPLSQETASDLAKLLPENNVLSPLPSQAMDDLMLSPDDIEQWFTEDPGPDEAPRMPEAAPPVAPAPAAPTPAAPAPAPSWPLSSSVPSQKTYQGSYGFRLGFLHSGTAKSVTCTYSPALNKMFCQLAKTCPVQLWVDSTPPPGTRVRAMAIYKQSQHMTEVVRRCPHHERCSDSDGLAPPQHLIRVEGNLRVEYLDDRNTFRHSVVVPYEPPEVGSDCTTIHYNYMCNSSCMGGMNRRPILTIITLEDSSGNLLGRNSFEVRVCACPGRDRRTEEENLRKKGEPHHELPPGSTKRALPNNTSSSPQPKKKPLDGEYFTLQIRGRERFEMFRELNEALELKDAQAGKEPGGSRAHSSHLKSKKGQSTSRHKKLMFKTEGPDSD

SEQ ID NO: 19 - protein, 393 aa, Homo sapiens; identical to SEQ ID NO: 16

SEQ ID NO: 20 - protein, 393 aa, Homo sapiens
MEEPQSDPSVEPPLSQETFSDLAKLAPENNVLSPLPSQAMDDLMLSPDDIEQWFTEDPGPDEAPRMPEAAPPVAPAPAAPTPAAPAPAPSWPLSSSVPSQKTYQGSYGFRLGFLHSGTAKSVTCTYSPALNKMFCQLAKTCPVQLWVDSTPPPGTRVRAMAIYKQSQHMTEVVRRCPHHERCSDSDGLAPPQHLIRVEGNLRVEYLDDRNTFRHSVVVPYEPPEVGSDCTTIHYNYMCNSSCMGGMNRRPILTIITLEDSSGNLLGRNSFEVRVCACPGRDRRTEEENLRKKGEPHHELPPGSTKRALPNNTSSSPQPKKKPLDGEYFTLQIRGRERFEMFRELNEALELKDAQAGKEPGGSRAHSSHLKSKKGQSTSRHKKLMFKTEGPDSD

SEQ ID NO: 21 - protein, 491 aa, Homo sapiens
MCNTNMSVPTDGAVTTSQIPASEQETLVRPKPLLLKLLKSVGAQKDTYTMKEVLFYLGQYIMTKRLYDEKQQHIVYCSNDLLGDLFGVPSFSVKEHRKIYTMIYRNLVVVNQQESSDSGTSVSENRCHLEGGSDQKDLVQELQEEKPSSSHLVSRPSTSSRRRAISETEENSDELSGERQRKRHKSDSISLSFDESLALCVIREICCERSSSSESTGTPSNPDLDAGVSEHSGDWLDQDSVSDQFSVEFEVESLDSEDYSLSEEGQELSDEDDEVYQVTVYQAGESDTDSFEEDPEISLADYWKCTSCNEMNPPLPSHCNRCWALRENWLPEDKGKDKGEISEKAKLENSTQAEEGFDVPDCKKTIVNDSRESCVEENDDKITQASQSQESEDYSQPSTSSSIIYSSQEDVKEFEREETQDKEESVESSLPLNAIEPCVICQGRPKNGCIVHGKTGHLMACFTCAKKLKKRNKPCPVCRQPIQMIVLTYFP

SEQ ID NO: 22 - protein, 324 aa, Homo sapiens
MSSEAETQQPPAAPPAAPALSAADTKPGTTGSGAGSGGPGGLTSAAPAGGDKKVIATKVLGTVKWFNVRNGYGFINRNDTKEDVFVHQTAIKKNNPRKYLRSVGDGETVEFDVVEGEKGAEAANVTGPGGVPVQGSKYAADRNHYRRYPRRRGPPRNYQQNYQNSESGEKNEGSESAPEGQAQQRRPYRRRRFPPYYMRRPYGRRPQYSNPPVQGEVMEGADNQGAGEQGRPVRQNMYRGYRPRFRRGPPRQRQPREDGNEEDKENQGDETQGQQPPQRRYRRNFNYRRRRPENPKPQDGKETKAADPPAENSSAPEAEQGGAE

SEQ ID NO: 23 - protein, 246 aa, Homo sapiens
MSSEAETQQPPAAPPAAPALSAADTKPGTTGSGAGSGGPGGLTSAAPAGGDGVPVQGSKYAADRNHYRRYPRRRGPPRNYQQNYQNSESGEKNEGSESAPEGQAQQRRPYRRRRFPPYYMRRPYGRRPQYSNPPVQGEVMEGADNQGAGEQGRPVRQNMYRGYRPRFRRGPPRQRQPREDGNEEDKENQGDETQGQQPPQRRYRRNFNYRRRRPENPKPQDGKETKAADPPAENSSAPEAEQGGAE